European Patent Application EP 4 130 257 A1, published February 8, 2023. Title: Improved Cytosine Base Editing System. Applicant: Suzhou Qi Biodesign Biotechnology Company Limited. Application EP EP 21764693.4. The sequence listing filed with the application follows.

SEQUENCE LISTING (40 sequences)

SEQ ID NO: 1 - protein, 10069 aa, artificial sequence
GAGCTCGGTACCTGACCCGGTCGTGCCCCTCTCTAGAGATAATGAGCATTGCATGTCTAAGTTATAAAAAATTACCACATATTTTTTTTGTCACACTTGTTTGAAGTGCAGTTTATCTATCTTTATACATATATTTAAACTTTACTCTACGAATAATATAATCTATAGTACTACAATAATATCAGTGTTTTAGAGAATCATATAAATGAACAGTTAGACATGGTCTAAAGGACAATTGAGTATTTTGACAACAGGACTCTACAGTTTTATCTTTTTAGTGTGCATGTGTTCTCCTTTTTTTTTGCAAATAGCTTCACCTATATAATACTTCATCCATTTTATTAGTACATCCATTTAGGGTTTAGGGTTAATGGTTTTTATAGACTAATTTTTTTAGTACATCTATTTTATTCTATTTTAGCCTCTAAATTAAGAAAACTAAAACTCTATTTTAGTTTTTTTATTTAATAATTTAGATATAAAATAGAATAAAATAAAGTGACTAAAAATTAAACAAATACCCTTTAAGAAATTAAAAAAACTAAGGAAACATTTTTCTTGTTTCGAGTAGATAATGCCAGCCTGTTAAACGCCGTCGACGAGTCTAACGGACACCAACCAGCGAACCAGCAGCGTCGCGTCGGGCCAAGCGAAGCAGACGGCACGGCATCTCTGTCGCTGCCTCTGGACCCCTCTCGATCGAGAGTTCCGCTCCACCGTTGGACTTGCTCCGCTGTCGGCATCCAGAAATTGCGTGGCGGAGCGGCAGACGTGAGCCGGCACGGCAGGCGGCCTCCTCCTCCTCTCACGGCACCGGCAGCTACGGGGGATTCCTTTCCCACCGCTCCTTCGCTTTCCCTTCCTCGCCCGCCGTAATAAATAGACACCCCCTCCACACCCTCTTTCCCCAACCTCGTGTTGTTCGGAGCGCACACACACACAACCAGATCTCCCCCAAATCCACCCGTCGGCACCTCCGCTTCAAGGTACGCCGCTCGTCCTCCCCCCCCCCCCCTCTCTACCTTCTCTAGATCGGCGTTCCGGTCCATGGTTAGGGCCCGGTAGTTCTACTTCTGTTCATGTTTGTGTTAGATCCGTGTTTGTGTTAGATCCGTGCTGCTAGCGTTCGTACACGGATGCGACCTGTACGTCAGACACGTTCTGATTGCTAACTTGCCAGTGTTTCTCTTTGGGGAATCCTGGGATGGCTCTAGCCGTTCCGCAGACGGGATCGATTTCATGATTTTTTTTGTTTCGTTGCATAGGGTTTGGTTTGCCCTTTTCCTTTATTTCAATATATGCCGTGCACTTGTTTGTCGGGTCATCTTTTCATGCTTTTTTTTGTCTTGGTTGTGATGATGTGGTCTGGTTGGGCGGTCGTTCTAGATCGGAGTAGAATTAATTCTGTTTCAAACTACCTGGTGGATTTATTAATTTTGGATCTGTATGTGTGTGCCATACATATTCATAGTTACGAATTGAAGATGATGGATGGAAATATCGATCTAGGATAGGTATACATGTTGATGCGGGTTTTACTGATGCATATACAGAGATGCTTTTTGTTCGCTTGGTTGTGATGATGTGGTGTGGTTGGGCGGTCGTTCATTCGTTCTAGATCGGAGTAGAATACTGTTTCAAACTACCTGGTGTATTTATTAATTTTGGAACTGTATGTGTGTGTCATACATCTTCATAGTTACGAGTTTAAGATGGATGGAAATATCGATCTAGGATAGGTATACATGTTGATGTGGGTTTTACTGATGCATATACATGATGGCATATGCAGCATCTATTCATATGCTCTAACCTTGAGTACCTATCTATTATAATAAACAAGTATGTTTTATAATTATTTTGATCTTGATATACTTGGATGATGGCATATGCAGCAGCTATATGTGGATTTTTTTAGCCCTGCCTTCATACGCTATTTATTTGCTTGGTACTGTTTCTTTTGTCGATGCTCACCCTGTTGTTTGGTGTTACTTCTGCAAAGCTTGTCGACGGATCCATGGAGGCCAGCCCGGCTAGCGGCCCAAGGCATCTCATGGACCCGCACATCTTCACCAGCAACTTCAACAACGGCATCGGCAGGCACAAGACCTACTTGTGCTACGAGGTGGAGAGGCTCGACAACGGAACCTCCGTGAAGATGGACCAACACAGGGGGTTCCTCCACAACCAAGCCAAGAACCTCCTCTGCGGCTTCTACGGCAGGCACGCCGAGTTGAGGTTCCTCGACTTGGTGCCATCCCTCCAACTCGATCCAGCCCAAATCTACCGCGTGACCTGGTTCATCTCCTGGTCCCCATGCTTCTCCTGGGGTTGCGCCGGCGAGGTTCGGGCTTTCCTCCAAGAAAACACCCACGTCCGCCTCCGCATTTTCGCCGCCAGGATCTATGATTACGACCCTCTCTACAAGGAGGCCCTCCAGATGCTGCGGGACGCCGGTGCTCAGGTGAGTATCATGACCTACGACGAGTTCAAGCACTGCTGGGACACCTTCGTTGACCACCAGGGCTGCCCATTCCAACCATGGGACGGTCTGGATGAACACAGCCAAGCCTTGTCCGGCAGGCTCCGGGCCATCCTCCAAAACCAGGGGAACTCCGGGAGCGAGACGCCAGGCACCTCCGAGTCGGCCACCCCAGAATCTCTTAAGGACAAGAAGTACTCGATCGGCCTCGCCATCGGGACGAACTCAGTTGGCTGGGCCGTGATCACCGACGAGTACAAGGTGCCCTCTAAGAAGTTCAAGGTCCTGGGGAACACCGACCGCCATTCCATCAAGAAGAACCTCATCGGCGCTCTCCTGTTCGACAGCGGGGAGACCGCTGAGGCTACGAGGCTCAAGAGAACCGCTAGGCGCCGGTACACGAGAAGGAAGAACAGGATCTGCTACCTCCAAGAGATTTTCTCCAACGAGATGGCCAAGGTTGACGATTCATTCTTCCACCGCCTGGAGGAGTCTTTCCTCGTGGAGGAGGATAAGAAGCACGAGCGGCATCCCATCTTCGGCAACATCGTGGACGAGGTTGCCTACCACGAGAAGTACCCTACGATCTACCATCTGCGGAAGAAGCTCGTGGACTCCACCGATAAGGCGGACCTCAGACTGATCTACCTCGCTCTGGCCCACATGATCAAGTTCCGCGGCCATTTCCTGATCGAGGGGGATCTCAACCCAGACAACAGCGATGTTGACAAGCTGTTCATCCAACTCGTGCAGACCTACAACCAACTCTTCGAGGAGAACCCGATCAACGCCTCTGGCGTGGACGCGAAGGCTATCCTGTCCGCGAGGCTCTCGAAGTCCAGGAGGCTGGAGAACCTGATCGCTCAGCTCCCAGGCGAGAAGAAGAACGGCCTGTTCGGGAACCTCATCGCTCTCAGCCTGGGGCTCACCCCGAACTTCAAGTCGAACTTCGATCTCGCTGAGGACGCCAAGCTGCAACTCTCCAAGGACACCTACGACGATGACCTCGATAACCTCCTGGCCCAGATCGGCGATCAATACGCGGACCTGTTCCTCGCTGCCAAGAACCTGTCGGACGCCATCCTCCTGTCAGATATCCTCCGCGTGAACACCGAGATCACGAAGGCTCCACTCTCTGCCTCCATGATCAAGCGCTACGACGAGCACCATCAGGATCTGACCCTCCTGAAGGCGCTGGTCCGCCAACAGCTCCCGGAGAAGTACAAGGAGATTTTCTTCGATCAGTCGAAGAACGGCTACGCTGGGTACATCGACGGCGGGGCCTCACAAGAGGAGTTCTACAAGTTCATCAAGCCAATCCTGGAGAAGATGGACGGCACGGAGGAGCTCCTGGTGAAGCTCAACAGGGAGGACCTCCTGCGGAAGCAGAGAACCTTCGATAACGGCAGCATCCCCCACCAAATCCATCTCGGGGAGCTGCACGCCATCCTGAGAAGGCAAGAGGACTTCTACCCTTTCCTCAAGGATAACCGGGAGAAGATCGAGAAGATCCTGACCTTCAGAATCCCATACTACGTCGGCCCTCTCGCGCGGGGGAACTCAAGATTCGCTTGGATGACCCGCAAGTCTGAGGAGACCATCACGCCGTGGAACTTCGAGGAGGTGGTGGACAAGGGCGCTAGCGCTCAGTCGTTCATCGAGAGGATGACCAACTTCGACAAGAACCTGCCCAACGAGAAGGTGCTCCCTAAGCACTCGCTCCTGTACGAGTACTTCACCGTCTACAACGAGCTCACGAAGGTGAAGTACGTCACCGAGGGCATGCGCAAGCCAGCGTTCCTGTCCGGGGAGCAGAAGAAGGCTATCGTGGACCTCCTGTTCAAGACCAACCGGAAGGTCACGGTTAAGCAACTCAAGGAGGACTACTTCAAGAAGATCGAGTGCTTCGATTCGGTCGAGATCAGCGGCGTTGAGGACCGCTTCAACGCCAGCCTCGGGACCTACCACGATCTCCTGAAGATCATCAAGGATAAGGACTTCCTGGACAACGAGGAGAACGAGGATATCCTGGAGGACATCGTGCTGACCCTCACGCTGTTCGAGGACAGGGAGATGATCGAGGAGCGCCTGAAGACGTACGCCCATCTCTTCGATGACAAGGTCATGAAGCAACTCAAGCGCCGGAGATACACCGGCTGGGGGAGGCTGTCCCGCAAGCTCATCAACGGCATCCGGGACAAGCAGTCCGGGAAGACCATCCTCGACTTCCTCAAGAGCGATGGCTTCGCCAACAGGAACTTCATGCAACTGATCCACGATGACAGCCTCACCTTCAAGGAGGATATCCAAAAGGCTCAAGTGAGCGGCCAGGGGGACTCGCTGCACGAGCATATCGCGAACCTCGCTGGCTCCCCCGCGATCAAGAAGGGCATCCTCCAGACCGTGAAGGTTGTGGACGAGCTCGTGAAGGTCATGGGCCGGCACAAGCCTGAGAACATCGTCATCGAGATGGCCAGAGAGAACCAAACCACGCAGAAGGGGCAAAAGAACTCTAGGGAGCGCATGAAGCGCATCGAGGAGGGCATCAAGGAGCTGGGGTCCCAAATCCTCAAGGAGCACCCAGTGGAGAACACCCAACTGCAGAACGAGAAGCTCTACCTGTACTACCTCCAGAACGGCAGGGATATGTACGTGGACCAAGAGCTGGATATCAACCGCCTCAGCGATTACGACGTCGATCATATCGTTCCCCAGTCTTTCCTGAAGGATGACTCCATCGACAACAAGGTCCTCACCAGGTCGGACAAGAACCGCGGCAAGTCAGATAACGTTCCATCTGAGGAGGTCGTTAAGAAGATGAAGAACTACTGGAGGCAGCTCCTGAACGCCAAGCTGATCACGCAAAGGAAGTTCGACAACCTCACCAAGGCTGAGAGAGGCGGGCTCTCAGAGCTGGACAAGGCCGGCTTCATCAAGCGGCAGCTGGTCGAGACCAGACAAATCACGAAGCACGTTGCGCAAATCCTCGACTCTCGGATGAACACGAAGTACGATGAGAACGACAAGCTGATCAGGGAGGTTAAGGTGATCACCCTGAAGTCTAAGCTCGTCTCCGACTTCAGGAAGGATTTCCAGTTCTACAAGGTTCGCGAGATCAACAACTACCACCATGCCCATGACGCTTACCTCAACGCTGTGGTCGGCACCGCTCTGATCAAGAAGTACCCAAAGCTGGAGTCCGAGTTCGTGTACGGGGACTACAAGGTTTACGATGTGCGCAAGATGATCGCCAAGTCGGAGCAAGAGATCGGCAAGGCTACCGCCAAGTACTTCTTCTACTCAAACATCATGAACTTCTTCAAGACCGAGATCACGCTGGCCAACGGCGAGATCCGGAAGAGACCGCTCATCGAGACCAACGGCGAGACGGGGGAGATCGTGTGGGACAAGGGCAGGGATTTCGCGACCGTCCGCAAGGTTCTCTCCATGCCCCAGGTGAACATCGTCAAGAAGACCGAGGTCCAAACGGGCGGGTTCTCAAAGGAGTCTATCCTGCCTAAGCGGAACAGCGACAAGCTCATCGCCAGAAAGAAGGACTGGGACCCAAAGAAGTACGGCGGGTTCGACAGCCCTACCGTGGCCTACTCGGTCCTGGTTGTGGCGAAGGTTGAGAAGGGCAAGTCCAAGAAGCTCAAGAGCGTGAAGGAGCTCCTGGGGATCACCATCATGGAGAGGTCCAGCTTCGAGAAGAACCCAATCGACTTCCTGGAGGCCAAGGGCTACAAGGAGGTGAAGAAGGACCTGATCATCAAGCTCCCGAAGTACTCTCTCTTCGAGCTGGAGAACGGCAGGAAGAGAATGCTGGCTTCCGCTGGCGAGCTCCAGAAGGGGAACGAGCTCGCGCTGCCAAGCAAGTACGTGAACTTCCTCTACCTGGCTTCCCACTACGAGAAGCTCAAGGGCAGCCCGGAGGACAACGAGCAAAAGCAGCTGTTCGTCGAGCAGCACAAGCATTACCTCGACGAGATCATCGAGCAAATCTCCGAGTTCAGCAAGCGCGTGATCCTCGCCGACGCGAACCTGGATAAGGTCCTCTCCGCCTACAACAAGCACCGGGACAAGCCCATCAGAGAGCAAGCGGAGAACATCATCCATCTCTTCACCCTGACGAACCTCGGCGCTCCTGCTGCTTTCAAGTACTTCGACACCACGATCGATCGGAAGAGATACACCTCCACGAAGGAGGTCCTGGACGCGACCCTCATCCACCAGTCGATCACCGGCCTGTACGAGACGAGGATCGACCTCTCACAACTCGGCGGGGATAAGAGACCCGCAGCAACCAAGAAGGCAGGGCAAGCAAAGAAGAAGAAGACGCGTGACTCCGGCGGCAGCACCAACCTGTCCGACATCATCGAGAAGGAGACGGGCAAGCAACTCGTGATCCAGGAGAGCATCCTCATGCTGCCAGAGGAGGTGGAGGAGGTCATCGGCAACAAGCCAGAGTCCGACATCCTGGTGCACACCGCCTACGACGAGTCCACCGACGAGAACGTCATGCTCCTGACCAGCGACGCCCCAGAGTACAAGCCATGGGCCCTCGTCATCCAGGACAGCAACGGGGAGAACAAGATCAAGATGCTGTCGGGGGGGAGCCCAAAGAAGAAGCGGAAGGTGTAGTGTACAAGTAACCCGGGAATTCGGTACGCTGAAATCACCAGTCTCTCTCTACAAATCTATCTCTCTCTATTTTCTCCATAAATAATGTGTGAGTAGTTTCCCGATAAGGGAAATTAGGGTTCTTATAGGGTTTCGCTCATGTGTTGAGCATATAAGAAACCCTTAGTATGTATTTGTATTTGTAAAATACTTCTATCAATAAAATTTCTAATTCCTAAAACCAAAATCCAGTACTAAAATCCAGATCTCCTAAAGTCCCTATAGATCTTTGTCGTGAATATAAACCAGACACGAGACGACTAAACCTGGAGCCCAGACGCCGTTCGAAGCTAGAAGTACCGCTTAGGCAGGAGGCCGTTAGGGAAAAGATGCTAAGGCAGGGTTGGTTACGTTGACTCCCCCGTAGGTTTGGTTTAAATATGATGAAGTGGACGGAAGGAAGGAGGAAGACAAGGAAGGATAAGGTTGCAGGCCCTGTGCAAGGTAAGAAGATGGAAATTTGATAGAGGTACGCTACTATACTTATACTATACGCTAAGGGAATGCTTGTATTTATACCCTATACCCCCTAATAACCCCTTATCAATTTAAGAAATAATCCGCATAAGCCCCCGCTTAAAAATTGGTATCAGAGCCATGAATAGGTCTATGACCAAAACTCAAGAGGATAAAACCTCACCAAAATACGAAAGAGTTCTTAACTCTAAAGATAAAAGATCTTTCAAGATCAAAACTAGTTCCCTCACACCGGAGCATGCGATATCCTCGAGAGATCTAGGCGTAATCATGGTCATAGCTGTTTCCTGTGTGAAATTGTTATCCGCTCACAATTCCACACAACATACGAGCCGGAAGCATAAAGTGTAAAGCCTGGGGTGCCTAATGAGTGAGCTAACTCACATTAATTGCGTTGCGCTCACTGCCCGCTTTCCAGTCGGGAAACCTGTCGTGCCAGCTGCATTAATGAATCGGCCAACGCGCGGGGAGAGGCGGTTTGCGTATTGGGCGCTCTTCCGCTTCCTCGCTCACTGACTCGCTGCGCTCGGTCGTTCGGCTGCGGCGAGCGGTATCAGCTCACTCAAAGGCGGTAATACGGTTATCCACAGAATCAGGGGATAACGCAGGAAAGAACATGTGAGCAAAAGGCCAGCAAAAGGCCAGGAACCGTAAAAAGGCCGCGTTGCTGGCGTTTTTCCATAGGCTCCGCCCCCCTGACGAGCATCACAAAAATCGACGCTCAAGTCAGAGGTGGCGAAACCCGACAGGACTATAAAGATACCAGGCGTTTCCCCCTGGAAGCTCCCTCGTGCGCTCTCCTGTTCCGACCCTGCCGCTTACCGGATACCTGTCCGCCTTTCTCCCTTCGGGAAGCGTGGCGCTTTCTCAATGCTCACGCTGTAGGTATCTCAGTTCGGTGTAGGTCGTTCGCTCCAAGCTGGGCTGTGTGCACGAACCCCCCGTTCAGCCCGACCGCTGCGCCTTATCCGGTAACTATCGTCTTGAGTCCAACCCGGTAAGACACGACTTATCGCCACTGGCAGCAGCCACTGGTAACAGGATTAGCAGAGCGAGGTATGTAGGCGGTGCTACAGAGTTCTTGAAGTGGTGGCCTAACTACGGCTACACTAGAAGGACAGTATTTGGTATCTGCGCTCTGCTGAAGCCAGTTACCTTCGGAAAAAGAGTTGGTAGCTCTTGATCCGGCAAACAAACCACCGCTGGTAGCGGTGGTTTTTTTGTTTGCAAGCAGCAGATTACGCGCAGAAAAAAAGGATCTCAAGAAGATCCTTTGATCTTTTCTACGGGGTCTGACGCTCAGTGGAACGAAAACTCACGTTAAGGGATTTTGGTCATGAGATTATCAAAAAGGATCTTCACCTAGATCCTTTTAAATTAAAAATGAAGTTTTAAATCAATCTAAAGTATATATGAGTAAACTTGGTCTGACAGTTACCAATGCTTAATCAGTGAGGCACCTATCTCAGCGATCTGTCTATTTCGTTCATCCATAGTTGCCTGACTCCCCGTCGTGTAGATAACTACGATACGGGAGGGCTTACCATCTGGCCCCAGTGCTGCAATGATACCGCGAGACCCACGCTCACCGGCTCCAGATTTATCAGCAATAAACCAGCCAGCCGGAAGGGCCGAGCGCAGAAGTGGTCCTGCAACTTTATCCGCCTCCATCCAGTCTATTAATTGTTGCCGGGAAGCTAGAGTAAGTAGTTCGCCAGTTAATAGTTTGCGCAACGTTGTTGCCATTGCTACAGGCATCGTGGTGTCACGCTCGTCGTTTGGTATGGCTTCATTCAGCTCCGGTTCCCAACGATCAAGGCGAGTTACATGATCCCCCATGTTGTGCAAAAAAGCGGTTAGCTCCTTCGGTCCTCCGATCGTTGTCAGAAGTAAGTTGGCCGCAGTGTTATCACTCATGGTTATGGCAGCACTGCATAATTCTCTTACTGTCATGCCATCCGTAAGATGCTTTTCTGTGACTGGTGAGTACTCAACCAAGTCATTCTGAGAATAGTGTATGCGGCGACCGAGTTGCTCTTGCCCGGCGTCAATACGGGATAATACCGCGCCACATAGCAGAACTTTAAAAGTGCTCATCATTGGAAAACGTTCTTCGGGGCGAAAACTCTCAAGGATCTTACCGCTGTTGAGATCCAGTTCGATGTAACCCACTCGTGCACCCAACTGATCTTCAGCATCTTTTACTTTCACCAGCGTTTCTGGGTGAGCAAAAACAGGAAGGCAAAATGCCGCAAAAAAGGGAATAAGGGCGACACGGAAATGTTGAATACTCATACTCTTCCTTTTTCAATATTATTGAAGCATTTATCAGGGTTATTGTCTCATGAGCGGATACATATTTGAATGTATTTAGAAAAATAAACAAATAGGGGTTCCGCGCACATTTCCCCGAAAAGTGCCACCTGACGT

SEQ ID NO: 2 - protein, 196 aa, artificial sequence
EILRYLMDPDTFTFNFNNDPLVLRRRQTYLCYEVERLDNGTWVLMDQHMGFLCNEAKNLLCGFYGRHAELRFLDLVPSLQLDPAQIYRVTWFISWSPCFSWGCAGEVRAFLQENTHVRLRIFAARIYDYDPLYKEALQMLRDAGAQVSIMTYDEFEYCWDTFVYRQGCPFQPWDGLEEHSQALSGRLRAILQNQGN

SEQ ID NO: 3 - protein, 196 aa, artificial sequence
EILRYLMDPDTFTFNFNNDPLVLARRQTYLCYEVERLDNGTWVLMDQHMGFLCNEAKNLLCGFYGRHAELRFLDLVPSLQLDPAQIYRVTWFISWSPCFSWGCAGEVRAFLQENTHVRLRIFAARIYDYDPLYKEALQMLRDAGAQVSIMTYDEFEYCWDTFVYRQGCPFQPWDGLEEHSQALSGRLRAILQNQGN

SEQ ID NO: 4 - protein, 196 aa, artificial sequence
EILRYLMDPDTFTFNFNNDPLVLKRRQTYLCYEVERLDNGTWVLMDQHMGFLCNEAKNLLCGFYGRHAELRFLDLVPSLQLDPAQIYRVTWFISWSPCFSWGCAGEVRAFLQENTHVRLRIFAARIYDYDPLYKEALQMLRDAGAQVSIMTYDEFEYCWDTFVYRQGCPFQPWDGLEEHSQALSGRLRAILQNQGN

SEQ ID NO: 5 - protein, 196 aa, artificial sequence
EILRYLMDPDTFTFNFNNDPLVLRKRQTYLCYEVERLDNGTWVLMDQHMGFLCNEAKNLLCGFYGRHAELRFLDLVPSLQLDPAQIYRVTWFISWSPCFSWGCAGEVRAFLQENTHVRLRIFAARIYDYDPLYKEALQMLRDAGAQVSIMTYDEFEYCWDTFVYRQGCPFQPWDGLEEHSQALSGRLRAILQNQGN

SEQ ID NO: 6 - protein, 196 aa, artificial sequence
EILRYLMDPDTFTFNFNNDPLVLRRRQCYLCYEVERLDNGTWVLMDQHMGFLCNEAKNLLCGFYGRHAELRFLDLVPSLQLDPAQIYRVTWFISWSPCFSWGCAGEVRAFLQENTHVRLRIFAARIYDYDPLYKEALQMLRDAGAQVSIMTYDEFEYCWDTFVYRQGCPFQPWDGLEEHSQALSGRLRAILQNQGN

SEQ ID NO: 7 - protein, 196 aa, artificial sequence
EILRYLMDPDTFTFNFNNDPLVLRRRQGYLCYEVERLDNGTWVLMDQHMGFLCNEAKNLLCGFYGRHAELRFLDLVPSLQLDPAQIYRVTWFISWSPCFSWGCAGEVRAFLQENTHVRLRIFAARIYDYDPLYKEALQMLRDAGAQVSIMTYDEFEYCWDTFVYRQGCPFQPWDGLEEHSQALSGRLRAILQNQGN

SEQ ID NO: 8 - protein, 196 aa, artificial sequence
EILRYLMDPDTFTFNFNNDPLVLRRRQSYLCYEVERLDNGTWVLMDQHMGFLCNEAKNLLCGFYGRHAELRFLDLVPSLQLDPAQIYRVTWFISWSPCFSWGCAGEVRAFLQENTHVRLRIFAARIYDYDPLYKEALQMLRDAGAQVSIMTYDEFEYCWDTFVYRQGCPFQPWDGLEEHSQALSGRLRAILQNQGN

SEQ ID NO: 9 - protein, 196 aa, artificial sequence
EILRYLMDPDTFTFNFNNDPLVLRRRQVYLCYEVERLDNGTWVLMDQHMGFLCNEAKNLLCGFYGRHAELRFLDLVPSLQLDPAQIYRVTWFISWSPCFSWGCAGEVRAFLQENTHVRLRIFAARIYDYDPLYKEALQMLRDAGAQVSIMTYDEFEYCWDTFVYRQGCPFQPWDGLEEHSQALSGRLRAILQNQGN

SEQ ID NO: 10 - protein, 196 aa, artificial sequence
EILRYLMDPDTFTFNFNNDPLVLRRRQTYLCYEVERLDNGTWVKMDQHMGFLCNEAKNLLCGFYGRHAELRFLDLVPSLQLDPAQIYRVTWFISWSPCFSWGCAGEVRAFLQENTHVRLRIFAARIYDYDPLYKEALQMLRDAGAQVSIMTYDEFEYCWDTFVYRQGCPFQPWDGLEEHSQALSGRLRAILQNQGN

SEQ ID NO: 11 - protein, 196 aa, artificial sequence
EILRYLMDPDTFTFNFNNDPLVLRRRQTYLCYEVERLDNGTWVLMDQHMGFLCAEAKNLLCGFYGRHAELRFLDLVPSLQLDPAQIYRVTWFISWSPCFSWGCAGEVRAFLQENTHVRLRIFAARIYDYDPLYKEALQMLRDAGAQVSIMTYDEFEYCWDTFVYRQGCPFQPWDGLEEHSQALSGRLRAILQNQGN

SEQ ID NO: 12 - protein, 196 aa, artificial sequence
EILRYLMDPDTFTFNFNNDPLVLRRRQTYLCYEVERLDNGTWVLMDQHMGFLCNEAKNLLCGFYGRHAELRFLDLVPSLQLDPAQIYRVTWFISHSPCFSWGCAGEVRAFLQENTHVRLRIFAARIYDYDPLYKEALQMLRDAGAQVSIMTYDEFEYCWDTFVYRQGCPFQPWDGLEEHSQALSGRLRAILQNQGN

SEQ ID NO: 13 - protein, 196 aa, artificial sequence
EILRYLMDPDTFTFNFNNDPLVLRRRQTYLCYEVERLDNGTWVLMDQHMGFLCNEAKNLLCGFYGRHAELRFLDLVPSLQLDPAQIYRVTWFISWSPCFSWGCAGEVRAFLQENTHVRLRIKAARIYDYDPLYKEALQMLRDAGAQVSIMTYDEFEYCWDTFVYRQGCPFQPWDGLEEHSQALSGRLRAILQNQGN

SEQ ID NO: 14 - protein, 196 aa, artificial sequence
EILRYLMDPDTFTFNFNNDPLVLRRRQTYLCYEVERLDNGTWVLMDQHMGFLCNEAKNLLCGFYGRHAELRFLDLVPSLQLDPAQIYRVTWFISWSPCFSWGCAGEVRAFLQENTHVRLRIFAAKIYDYDPLYKEALQMLRDAGAQVSIMTYDEFEYCWDTFVYRQGCPFQPWDGLEEHSQALSGRLRAILQNQGN

SEQ ID NO: 15 - protein, 196 aa, artificial sequence
EILRYLMDPDTFTFNFNNDPLVLRRRQTYLCYEVERLDNGTWVLMDQHMGFLCNEAKNLLCGFYGRHAELRFLDLVPSLQLDPAQIYRVTWFISWSPCFSWGCAGEVRAFLQENTHVRLRIFAARIFDYDPLYKEALQMLRDAGAQVSIMTYDEFEYCWDTFVYRQGCPFQPWDGLEEHSQALSGRLRAILQNQGN

SEQ ID NO: 16 - protein, 196 aa, artificial sequence
EILRYLMDPDTFTFNFNNDPLVLRRRQTYLCYEVERLDNGTWVLMDQHMGFLCNEAKNLLCGFYGRHAELRFLDLVPSLQLDPAQIYRVTWFISWSPCFSWGCAGEVRAFLQENTHVRLRIFAARIYRYDPLYKEALQMLRDAGAQVSIMTYDEFEYCWDTFVYRQGCPFQPWDGLEEHSQALSGRLRAILQNQGN

SEQ ID NO: 17 - protein, 196 aa, artificial sequence
EILRYLMDPDTFTFNFNNDPLVLRRRQTYLCYEVERLDNGTWVLMDQHMGFLCNEAKNLLCGFYGRHAELRFLDLVPSLQLDPAQIYRVTWFISWSPCFSWGCAGEVRAFLQENTHVRLRIFAARIYHYDPLYKEALQMLRDAGAQVSIMTYDEFEYCWDTFVYRQGCPFQPWDGLEEHSQALSGRLRAILQNQGN

SEQ ID NO: 18 - protein, 196 aa, artificial sequence
EILRYLMDPDTFTFNFNNDPLVLRRRQTYLCYEVERLDNGTWVLMDQHMGFLCNEAKNLLCGFYGRHAELRFLDLVPSLQLDPAQIYRVTWFISWSPCFSWGCAGEVRAFLQENTHVRLRIFAARIYDMDPLYKEALQMLRDAGAQVSIMTYDEFEYCWDTFVYRQGCPFQPWDGLEEHSQALSGRLRAILQNQGN

SEQ ID NO: 19 - protein, 382 aa, artificial sequence
MNPQIRNPMERMYRDTFYDNFENEPILYGRSYTWLCYEVKIKRGRSNLLWDTGVFRGQVYFKPQYHAEMCFLSWFCGNQLPAYKCFQITWFVSWTPCPDCVAKLAEFLSEHPNVTLTISAARLYYYWERDYRRALCRLSQAGARVKIMDYEEFAYCWENFVYNEGQQFMPWYKFDENYAFLHRTLKEILRYLMDPDTFTFNFNNDPLVLRRRQTYLCYEVERLDNGTWVLMDQHMGFLCNEAKNLLCGFYGRHAELRFLDLVPSLQLDPAQIYRVTWFISWSPCFSWGCAGEVRAFLQENTHVRLRIFAARIYDYDPLYKEALQMLRDAGAQVSIMTYDEFEYCWDTFVYRQGCPFQPWDGLEEHSQALSGRLRAILQNQGN

SEQ ID NO: 20 - protein, 199 aa, artificial sequence
MEASPASGPRHLMDPHIFTSNFNNGIGRHKTYLCYEVERLDNGTSVKMDQHRGFLHNQAKNLLCGFYGRHAELRFLDLVPSLQLDPAQIYRVTWFISWSPCFSWGCAGEVRAFLQENTHVRLRIFAARIYDYDPLYKEALQMLRDAGAQVSIMTYDEFKHCWDTFVDHQGCPFQPWDGLDEHSQALSGRLRAILQNQGN

SEQ ID NO: 21 - protein, 228 aa, artificial sequence
SSETGPVAVDPTLRRRIEPHEFEVFFDPRELRKETCLLYEINWGGRHSIWRHTSQNTNKHVEVNFIEKFTTERYFCPNTRCSITWFLSYSPCGECSRAITEFLSRYPHVTLFIYIARLYHHADPENRQGLEDLISSGVTIQIMTEQESGYCWRNFVNYSPSNEAHWPRYPHLWVRLYVLELYCIILGLPPCLNILRRKQPQLTFFTIALQSCHYQRLPPHILWATGLK

SEQ ID NO: 22 - protein, 228 aa, artificial sequence
SSETGPVAVDPTLRRRIEPHEFEVFFDPRELAAETCLLYEINWGGRHSIWRHTSQNTNKHVEVNFIEKFTTERYFCPNTRCSITWFLSWSPCGECSRAITEFLSRYPHVTLFIYIARLYHHADPRNRQGLRDLISSGVTIQIMTEQESGYCWRNFVNYSPSNEAHWPRYPHLWVRLYVLELYCIILGLPPCLNILRRKQPQLTFFTIALQSCHYQRLPPHILWATGLK

SEQ ID NO: 23 - protein, 199 aa, artificial sequence
MEASPASGPRHLMDPHIFTSNFNNGIGRHKTYLCYEVERLDNGTSVKMDQHRGFLHGQAKNLLCGFYGRHAELRFLDLVPSLQLDPAQIYRVTWFISWSPCFSWGCAGEVRAFLQENTHVRLRIFAARIYDYDPLYKEALQMLRDAGAQVSIMTYDEFKHCWDTFVDHQGCPFQPWDGLDEHSQALSGRLRAILQNQGN

SEQ ID NO: 24 - protein, 199 aa, artificial sequence
MEASPASGPRHLMDPHIFTSNFNNGIGRHKTYLCYEVERLDNGTSVKMDQHRGFLHNQAKNLLCGFYGRHAELRFLDLVPSLQLDPAQIYRVTWFISWSPCFSWGCAGEVRAFLQENTHVRLRIFAAAIYDYDPLYKEALQMLRDAGAQVSIMTYDEFKHCWDTFVDHQGCPFQPWDGLDEHSQALSGRLRAILQNQGN

SEQ ID NO: 25 - protein, 199 aa, artificial sequence
MEASPASGPRHLMDPHIFTSNFNNGIGRHKTYLCYEVERLDNGTSVKMDQHRGFLHNQAKNLLCGFYGRHAELRFLDLVPSLQLDPAQIYRVTWFISWSPCFSWGCAGEVRAFLQENTHVRLRIFAARIFDYDPLYKEALQMLRDAGAQVSIMTYDEFKHCWDTFVDHQGCPFQPWDGLDEHSQALSGRLRAILQNQGN

SEQ ID NO: 26 - protein, 196 aa, artificial sequence
EILRYLMDPDTFTFNFNNDPLVLRKRQTYLCYEVERLDNGTWVLMDQHMGFLCNEAKNLLCGFYGRHAELRFLDLVPSLQLDPAQIYRVTWFISWSPCFSWGCAGEVRAFLQENTHVRLRIFAAKIYDYDPLYKEALQMLRDAGAQVSIMTYDEFEYCWDTFVYRQGCPFQPWDGLEEHSQALSGRLRAILQNQGN

SEQ ID NO: 27 - protein, 196 aa, artificial sequence
EILRYLMDPDTFTFNFNNDPLVLRKRQTYLCYEVERLDNGTWVLMDQHMGFLCNEAKNLLCGFYGRHAELRFLDLVPSLQLDPAQIYRVTWFISWSPCFSWGCAGEVRAFLQENTHVRLRIFAARIFDYDPLYKEALQMLRDAGAQVSIMTYDEFEYCWDTFVYRQGCPFQPWDGLEEHSQALSGRLRAILQNQGN

SEQ ID NO: 28 - protein, 196 aa, artificial sequence
EILRYLMDPDTFTFNFNNDPLVLRKRQTYLCYEVERLDNGTWVLMDQHMGFLCNEAKNLLCGFYGRHAELRFLDLVPSLQLDPAQIYRVTWFISWSPCFSWGCAGEVRAFLQENTHVRLRIFAARIYRYDPLYKEALQMLRDAGAQVSIMTYDEFEYCWDTFVYRQGCPFQPWDGLEEHSQALSGRLRAILQNQGN

SEQ ID NO: 29 - protein, 196 aa, artificial sequence
EILRYLMDPDTFTFNFNNDPLVLRRRQTYLCYEVERLDNGTWVLMDQHMGFLCNEAKNLLCGFYGRHAELRFLDLVPSLQLDPAQIYRVTWFISWSPCFSWGCAGEVRAFLQENTHVRLRIFAAKIFDYDPLYKEALQMLRDAGAQVSIMTYDEFEYCWDTFVYRQGCPFQPWDGLEEHSQALSGRLRAILQNQGN

SEQ ID NO: 30 - protein, 196 aa, artificial sequence
EILRYLMDPDTFTFNFNNDPLVLRRRQVYLCYEVERLDNGTWVLMDQHMGFLCNEAKNLLCGFYGRHAELRFLDLVPSLQLDPAQIYRVTWFISWSPCFSWGCAGEVRAFLQENTHVRLRIFAARIYRYDPLYKEALQMLRDAGAQVSIMTYDEFEYCWDTFVYRQGCPFQPWDGLEEHSQALSGRLRAILQNQGN

SEQ ID NO: 31 - protein, 196 aa, artificial sequence
EILRYLMDPDTFTFNFNNDPLVLRRRQTYLCYEVERLDNGTWVLMDQHMGFLCNEAKNLLCGFYGRHAELRFLDLVPSLQLDPAQIYRVTWFISWSPCFSWGCAGEVRAFLQENTHVRLRIFAARIYRMDPLYKEALQMLRDAGAQVSIMTYDEFEYCWDTFVYRQGCPFQPWDGLEEHSQALSGRLRAILQNQGN

SEQ ID NO: 32 - protein, 196 aa, artificial sequence
EILRYLMDPDTFTFNFNNDPLVLRKRQTYLCYEVERLDNGTWVLMDQHMGFLCNEAKNLLCGFYGRHAELRFLDLVPSLQLDPAQIYRVTWFISWSPCFSWGCAGEVRAFLQENTHVRLRIFAAKIYRYDPLYKEALQMLRDAGAQVSIMTYDEFEYCWDTFVYRQGCPFQPWDGLEEHSQALSGRLRAILQNQGN

SEQ ID NO: 33 - protein, 196 aa, artificial sequence
EILRYLMDPDTFTFNFNNDPLVLRKRQVYLCYEVERLDNGTWVLMDQHMGFLCNEAKNLLCGFYGRHAELRFLDLVPSLQLDPAQIYRVTWFISWSPCFSWGCAGEVRAFLQENTHVRLRIFAARIFDYDPLYKEALQMLRDAGAQVSIMTYDEFEYCWDTFVYRQGCPFQPWDGLEEHSQALSGRLRAILQNQGN

SEQ ID NO: 34 - protein, 196 aa, artificial sequence
EILRYLMDPDTFTFNFNNDPLVLRRRQVYLCYEVERLDNGTWVLMDQHMGFLCNEAKNLLCGFYGRHAELRFLDLVPSLQLDPAQIYRVTWFISWSPCFSWGCAGEVRAFLQENTHVRLRIFAARIYHMDPLYKEALQMLRDAGAQVSIMTYDEFEYCWDTFVYRQGCPFQPWDGLEEHSQALSGRLRAILQNQGN

SEQ ID NO: 35 - protein, 1369 aa, artificial sequence
LKDKKYSIGLAIGTNSVGWAVITDEYKVPSKKFKVLGNTDRHSIKKNLIGALLFDSGETAEATRLKRTARRRYTRRKNRICYLQEIFSNEMAKVDDSFFHRLEESFLVEEDKKHERHPIFGNIVDEVAYHEKYPTIYHLRKKLVDSTDKADLRLIYLALAHMIKFRGHFLIEGDLNPDNSDVDKLFIQLVQTYNQLFEENPINASGVDAKAILSARLSKSRRLENLIAQLPGEKKNGLFGNLIALSLGLTPNFKSNFDLAEDAKLQLSKDTYDDDLDNLLAQIGDQYADLFLAAKNLSDAILLSDILRVNTEITKAPLSASMIKRYDEHHQDLTLLKALVRQQLPEKYKEIFFDQSKNGYAGYIDGGASQEEFYKFIKPILEKMDGTEELLVKLNREDLLRKQRTFDNGSIPHQIHLGELHAILRRQEDFYPFLKDNREKIEKILTFRIPYYVGPLARGNSRFAWMTRKSEETITPWNFEEVVDKGASAQSFIERMTNFDKNLPNEKVLPKHSLLYEYFTVYNELTKVKYVTEGMRKPAFLSGEQKKAIVDLLFKTNRKVTVKQLKEDYFKKIECFDSVEISGVEDRFNASLGTYHDLLKIIKDKDFLDNEENEDILEDIVLTLTLFEDREMIEERLKTYAHLFDDKVMKQLKRRRYTGWGRLSRKLINGIRDKQSGKTILDFLKSDGFANRNFMQLIHDDSLTFKEDIQKAQVSGQGDSLHEHIANLAGSPAIKKGILQTVKVVDELVKVMGRHKPENIVIEMARENQTTQKGQKNSRERMKRIEEGIKELGSQILKEHPVENTQLQNEKLYLYYLQNGRDMYVDQELDINRLSDYDVDHIVPQSFLKDDSIDNKVLTRSDKNRGKSDNVPSEEVVKKMKNYWRQLLNAKLITQRKFDNLTKAERGGLSELDKAGFIKRQLVETRQITKHVAQILDSRMNTKYDENDKLIREVKVITLKSKLVSDFRKDFQFYKVREINNYHHAHDAYLNAVVGTALIKKYPKLESEFVYGDYKVYDVRKMIAKSEQEIGKATAKYFFYSNIMNFFKTEITLANGEIRKRPLIETNGETGEIVWDKGRDFATVRKVLSMPQVNIVKKTEVQTGGFSKESILPKRNSDKLIARKKDWDPKKYGGFDSPTVAYSVLVVAKVEKGKSKKLKSVKELLGITIMERSSFEKNPIDFLEAKGYKEVKKDLIIKLPKYSLFELENGRKRMLASAGELQKGNELALPSKYVNFLYLASHYEKLKGSPEDNEQKQLFVEQHKHYLDEIIEQISEFSKRVILADANLDKVLSAYNKHRDKPIREQAENIIHLFTLTNLGAPAAFKYFDTTIDRKRYTSTKEVLDATLIHQSITGLYETRIDLSQLGGD

SEQ ID NO: 36 - protein, 16 aa, artificial sequence
SGSETPGTSESATPES

SEQ ID NO: 37 - protein, 32 aa, artificial sequence
SGGSSGGSSGSETPGTSESATPESSGGSSGGS

SEQ ID NO: 38 - protein, 90 aa, artificial sequence
TRDSGGSTNLSDIIEKETGKQLVIQESILMLPEEVEEVIGNKPESDILVHTAYDESTDENVMLLTSDAPEYKPWALVIQDSNGENKIKML

SEQ ID NO: 39 - protein, 7 aa, artificial sequence
PKKKRKV

SEQ ID NO: 40 - protein, 16 aa, artificial sequence
KRPAATKKAGQAKKKK